European Patent Application EP 4 692 351 A1, published February 11, 2026. Title: ANTI-CD25 ANTIBODY AND DRUG CONJUGATE THEREOF. Applicant: Daiichi Sankyo Company, Limited. Application JP. The sequence listing filed with the application follows.

SEQUENCE LISTING (58 sequences)

SEQ ID NO: 1 - protein, 6 aa, Rattus norvegicus
ESVSTR

SEQ ID NO: 2 - skipped

SEQ ID NO: 3 - protein, 8 aa, Rattus norvegicus
QQSWNGWA

SEQ ID NO: 4 - protein, 11 aa, Rattus norvegicus
QSLSHTNGNTY

SEQ ID NO: 5 - skipped

SEQ ID NO: 6 - protein, 9 aa, Rattus norvegicus
VQSTHVPNT

SEQ ID NO: 7 - protein, 8 aa, Rattus norvegicus
GFTFNNYY

SEQ ID NO: 8 - protein, 8 aa, Rattus norvegicus
ISTGGGTT

SEQ ID NO: 9 - protein, 20 aa, Rattus norvegicus
TTSVYFSDGSSHYDGEWFAY

SEQ ID NO: 10 - protein, 8 aa, Rattus norvegicus
GYTFTDYW

SEQ ID NO: 11 - protein, 8 aa, Rattus norvegicus
IYPNSGAT

SEQ ID NO: 12 - protein, 7 aa, Rattus norvegicus
TTYDFDY

SEQ ID NO: 13 - protein, 233 aa, Homo sapiens
MVLQTQVFISLLLWISGAYGDIVMTQSPDSLAVSLGERATINCKASESVSTRMHWYQQKPGQPPKLLIYKASNLASGVPARFSGSGSGTDFTLTISSLQAEDVAVYYCQQSWNGWAFGQGTKVEIKRTVAAPSVFIFPPSDEQLKSGTASVVCLLNNFYPREAKVQWKVDNALQSGNSQESVTEQDSKDSTYSLSSTLTLSKADYEKHKVYACEVTHQGLSSPVTKSFNRGEC

SEQ ID NO: 14 - protein, 233 aa, Homo sapiens
MVLQTQVFISLLLWISGAYGEIVLTQSPGTLSLSPGERATLSCKASESVSTRMHWYQQKPGQAPRLLIYKASNLASGVPARFSGSGSGTDFTLTISRLEPEDFAVYFCQQSWNGWAFGQGTKVEIKRTVAAPSVFIFPPSDEQLKSGTASVVCLLNNFYPREAKVQWKVDNALQSGNSQESVTEQDSKDSTYSLSSTLTLSKADYEKHKVYACEVTHQGLSSPVTKSFNRGEC

SEQ ID NO: 15 - protein, 476 aa, Homo sapiens
MKHLWFFLLLVAAPRWVLSEVQLVESGGGLVQPGGSLRLSCAASGFTFNNYYMVWVRQAPGKGLEWVAYISTGGGTTYYRESVKGRFTISRDNSKSTLYLQMNSLRAEDTAVYYCTTSVYFSDGSSHYDGEWFAYWGQGTLVTVSSASTKGPSVFPLAPSSKSTSGGTAALGCLVKDYFPEPVTVSWNSGALTSGVHTFPAVLQSSGLYSLSSVVTVPSSSLGTQTYICNVNHKPSNTKVDKKVEPKSCDKTHTCPPCPAPELLGGPSVFLFPPKPKDTLMISRTPEVTCVVVDVSHEDPEVKFNWYVDGVEVHNAKTKPREEQYNSTYRVVSVLTVLHQDWLNGKEYKCKVSNKALPAPIEKTISKAKGQPREPQVYTLPPSREEMTKNQVSLTCLVKGFYPSDIAVEWESNGQPENNYKTTPPVLDSDGSFFLYSKLTVDKSRWQQGNVFSCSVMHEALHNHYTQKSLSLSPGK

SEQ ID NO: 16 - protein, 476 aa, Homo sapiens
MKHLWFFLLLVAAPRWVLSEVQLVESGGGLVQPGGSLRLSCAASGFTFNNYYMVWVRQAPGKGLEWVAYISTGGGTTYYADSVKGRFTISRDNSKSTLYLQMNSLRAEDTAVYYCTTSVYFSDGSSHYDGEWFAYWGQGTLVTVSSASTKGPSVFPLAPSSKSTSGGTAALGCLVKDYFPEPVTVSWNSGALTSGVHTFPAVLQSSGLYSLSSVVTVPSSSLGTQTYICNVNHKPSNTKVDKKVEPKSCDKTHTCPPCPAPELLGGPSVFLFPPKPKDTLMISRTPEVTCVVVDVSHEDPEVKFNWYVDGVEVHNAKTKPREEQYNSTYRVVSVLTVLHQDWLNGKEYKCKVSNKALPAPIEKTISKAKGQPREPQVYTLPPSREEMTKNQVSLTCLVKGFYPSDIAVEWESNGQPENNYKTTPPVLDSDGSFFLYSKLTVDKSRWQQGNVFSCSVMHEALHNHYTQKSLSLSPGK

SEQ ID NO: 17 - protein, 272 aa, Homo sapiens
MDSYLLMWGLLTFIMVPGCQAELCDDDPPEIPHATFKAMAYKEGTMLNCECKRGFRRIKSGSLYMLCTGNSSHSSWDNQCQCTSSATRNTTKQVTPQPEEQKERKTTEMQSPMQPVDQASLPGHCREPPPWENEATERIYHFVVGQMVYYQCVQGYRALHRGPAESVCKMTHGKTRWTQPQLICTGEMETSQFPGEEKPQASPEGRPESETSCLVTTTDFQIQTEMAATMETSIFTTEYQVAVAGCVFLLISVLLLSGLTWQRRQRKSRRTI

SEQ ID NO: 18 - protein, 106 aa, Rattus norvegicus
DTVLTQSPALAVSPGERVTISCKASESVSTRMHWYQQKPGQQPKLLIYKASNLASGVPARFSGSGSGTDFTLTIDPVEADDTATYFCQQSWNGWAFGGGTKLELKR

SEQ ID NO: 19 - DNA, 318 bp, Rattus norvegicus
  source 1..318: mol_type = other DNA
gacactgtgctgacccagtctcctgctttggctgtgtctccaggagagagggttaccatctcctgtaaggccagtgaaagtgtcagtacacgtatgcactggtaccaacagaaaccaggacagcaacccaaactcctcatctataaagcatcaaacctagcatctggggtccctgccaggttcagtggcagtgggtctgggacagacttcaccctcaccattgatcctgtggaggctgatgacactgcaacctatttctgtcagcagagttggaatggttgggcgttcggtggaggcaccaagctggaattgaaacgg

SEQ ID NO: 20 - protein, 127 aa, Rattus norvegicus
EVQLVESGGGLVQPGRSLKLSCAASGFTFNNYYMVWVRQAPTKGLEWVAYISTGGGTTYYRESVKGRFTISRDNAKSTLYLQMDSLRSEDTATYYCTTSVYFSDGSSHYDGEWFAYWGQGTLVTVSS

SEQ ID NO: 21 - DNA, 381 bp, Rattus norvegicus
  source 1..381: mol_type = other DNA
gaggtgcagctggtggaatctgggggaggcttagtgcagcctggaaggtccctgaaactctcctgtgcagcctcaggattcactttcaataactattacatggtctgggtccgccaggctccaacgaagggtctggagtgggtcgcatacattagtactggtggtggtaccacttactatcgagagtccgtgaagggccggttcactatctccagagataatgcaaaaagcaccctatacctgcagatggacagtctgaggtctgaagacacggccacttattactgtacaacgagtgtttatttttctgatggtagttctcactacgatggggagtggtttgcttactggggccaaggcactctggtcactgtctcttca

SEQ ID NO: 22 - protein, 113 aa, Rattus norvegicus
DVVLTQTPPTLSATIGQSVSISCRSSQSLSHTNGNTYLYWLLQRPGQPPQLLIYFVSRLESGVPNRFSGSGSGTDFTLKISGVEAEDLGLYYCVQSTHVPNTFGAGTKLELKR

SEQ ID NO: 23 - DNA, 339 bp, Rattus norvegicus
  source 1..339: mol_type = other DNA
gatgttgtgctgacccagactccacccactttatcggctaccattggacaatcagtctccatctcttgcaggtcaagtcagagtctctcacatactaatggaaacacctatttatattggttgctacagaggccaggccaacctccacaacttctaatttatttcgtgtccaggcttgaatctggggtccccaacaggttcagtggcagtgggtcaggaactgatttcacactcaaaatcagtggagtagaggctgaggatttgggactttattactgcgtgcaaagtacccatgttccgaacacgtttggagctgggaccaagctggaactgaaacgg

SEQ ID NO: 24 - protein, 114 aa, Rattus norvegicus
QVKLLQSGAALEKPGASVKMSCKASGYTFTDYWVIWVKQSHGKSLEWIGEIYPNSGATNFNAKFKGKATLTVDKSTSTAYMELSRLTSEDSAIYYCTTYDFDYWGQGVMVTVSS

SEQ ID NO: 25 - DNA, 342 bp, Rattus norvegicus
  source 1..342: mol_type = other DNA
caggtcaagttgctgcagtctggggctgcactggagaagcctggagcctctgtgaagatgtcttgcaaagcttctggttatacattcactgactactgggtgatctgggtgaagcagagtcatggaaagagccttgagtggattggggaaatttatcctaacagtggtgctactaacttcaatgcaaagttcaagggcaaggccacattgactgtagacaaatccaccagcacagcctatatggagctcagcagattgacatctgaggactctgcaatctattactgtacaacatacgactttgattattggggccaaggagtcatggtcacagtctcctca

SEQ ID NO: 26 - protein, 232 aa, synthetic construct
MVLQTQVFISLLLWISGAYGDTVLTQSPALAVSPGERVTISCKASESVSTRMHWYQQKPGQQPKLLIYKASNLASGVPARFSGSGSGTDFTLTIDPVEADDTATYFCQQSWNGWAFGGGTKLELKRTVAAPSVFIFPPSDEQLKSGTASVVCLLNNFYPREAKVQWKVDNALQSGNSQESVTEQDSKDSTYSLSSTLTLSKADYEKHKVYACEVTHQGLSSPVTKSFNRGEC

SEQ ID NO: 27 - protein, 476 aa, synthetic construct
MKHLWFFLLLVAAPRWVLSEVQLVESGGGLVQPGRSLKLSCAASGFTFNNYYMVWVRQAPTKGLEWVAYISTGGGTTYYRESVKGRFTISRDNAKSTLYLQMDSLRSEDTATYYCTTSVYFSDGSSHYDGEWFAYWGQGTLVTVSSASTKGPSVFPLAPSSKSTSGGTAALGCLVKDYFPEPVTVSWNSGALTSGVHTFPAVLQSSGLYSLSSVVTVPSSSLGTQTYICNVNHKPSNTKVDKRVEPKSCDKTHTCPPCPAPEAAGGPSVFLFPPKPKDTLMISRTPEVTCVVVDVSHEDPEVKFNWYVDGVEVHNAKTKPREEQYNSTYRVVSVLTVLHQDWLNGKEYKCKVSNKALPAPIEKTISKAKGQPREPQVYTLPPSREEMTKNQVSLTCLVKGFYPSDIAVEWESNGQPENNYKTTPPVLDSDGSFFLYSKLTVDKSRWQQGNVFSCSVMHEALHNHYTQKSLSLSPGK

SEQ ID NO: 28 - DNA, 696 bp, synthetic construct
  source 1..696: mol_type = other DNA
atggtgctgcagacccaggtgttcatctccctgctgctgtggatctccggcgcgtacggcgacactgtgctgacccagtctcctgctttggctgtgtctccaggagagagggttaccatctcctgtaaggccagtgaaagtgtcagtacacgtatgcactggtaccaacagaaaccaggacagcaacccaaactcctcatctataaagcatcaaacctagcatctggggtccctgccaggttcagtggcagtgggtctgggacagacttcaccctcaccattgatcctgtggaggctgatgacactgcaacctatttctgtcagcagagttggaatggttgggcgttcggtggaggcaccaagctggaattgaaacggacggtggccgccccctccgtgttcatcttccccccctccgacgagcagctgaagtccggcaccgcctccgtggtgtgcctgctgaataacttctaccccagagaggccaaggtgcagtggaaggtggacaacgccctgcagtccgggaactcccaggagagcgtgaccgagcaggacagcaaggacagcacctacagcctgagcagcaccctgaccctgagcaaagccgactacgagaagcacaaggtgtacgcctgcgaggtgacccaccagggcctgagctcccccgtcaccaagagcttcaacaggggggagtgt

SEQ ID NO: 29 - DNA, 1428 bp, synthetic construct
  source 1..1428: mol_type = other DNA
atgaaacacctgtggttcttcctcctgctggtggcagctcccagatgggtgctgagcgaggtgcagctggtggaatctgggggaggcttagtgcagcctggaaggtccctgaaactctcctgtgcagcctcaggattcactttcaataactattacatggtctgggtccgccaggctccaacgaagggtctggagtgggtcgcatacattagtactggtggtggtaccacttactatcgagagtccgtgaagggccggttcactatctccagagataatgcaaaaagcaccctatacctgcagatggacagtctgaggtctgaagacacggccacttattactgtacaacgagtgtttatttttctgatggtagttctcactacgatggggagtggtttgcttactggggccaaggcactctggtcactgtcagctcagcctccaccaagggcccaagcgtcttccccctggcaccctcctccaagagcacctctggcggcacagccgccctgggctgcctggtcaaggactacttccccgaacccgtgaccgtgagctggaactcaggcgccctgaccagcggcgtgcacaccttccccgctgtcctgcagtcctcaggactctactccctcagcagcgtggtgaccgtgccctccagcagcttgggcacccagacctacatctgcaacgtgaatcacaagcccagcaacaccaaggtggacaagagagttgagcccaaatcttgtgacaaaactcacacatgcccaccctgcccagcacctgaagccgcggggggaccctcagtcttcctcttccccccaaaacccaaggacaccctcatgatctcccggacccctgaggtcacatgcgtggtggtggacgtgagccacgaagaccctgaggtcaagttcaactggtacgtggacggcgtggaggtgcataatgccaagacaaagccccgggaggagcagtacaacagcacgtaccgggtggtcagcgtcctcaccgtcctgcaccaggactggctgaatggcaaggagtacaagtgcaaggtctccaacaaagccctcccagcccccatcgagaaaaccatctccaaagccaaaggccagccccgggaaccacaggtgtacaccctgcccccatcccgggaggagatgaccaagaaccaggtcagcctgacctgcctggtcaaaggcttctatcccagcgacatcgccgtggagtgggagagcaatggccagcccgagaacaactacaagaccacccctcccgtgctggactccgacggctccttcttcctctacagcaagctcaccgtggacaagagcaggtggcagcagggcaacgtcttctcatgctccgtgatgcatgaggctctgcacaaccactacacccagaagagcctctccctgtctcccggcaaa

SEQ ID NO: 30 - protein, 239 aa, synthetic construct
MVLQTQVFISLLLWISGAYGDVVLTQTPPTLSATIGQSVSISCRSSQSLSHTNGNTYLYWLLQRPGQPPQLLIYFVSRLESGVPNRFSGSGSGTDFTLKISGVEAEDLGLYYCVQSTHVPNTFGAGTKLELKRTVAAPSVFIFPPSDEQLKSGTASVVCLLNNFYPREAKVQWKVDNALQSGNSQESVTEQDSKDSTYSLSSTLTLSKADYEKHKVYACEVTHQGLSSPVTKSFNRGEC

SEQ ID NO: 31 - protein, 463 aa, synthetic construct
MKHLWFFLLLVAAPRWVLSQVKLLQSGAALEKPGASVKMSCKASGYTFTDYWVIWVKQSHGKSLEWIGEIYPNSGATNFNAKFKGKATLTVDKSTSTAYMELSRLTSEDSAIYYCTTYDFDYWGQGVMVTVSSASTKGPSVFPLAPSSKSTSGGTAALGCLVKDYFPEPVTVSWNSGALTSGVHTFPAVLQSSGLYSLSSVVTVPSSSLGTQTYICNVNHKPSNTKVDKRVEPKSCDKTHTCPPCPAPEAAGGPSVFLFPPKPKDTLMISRTPEVTCVVVDVSHEDPEVKFNWYVDGVEVHNAKTKPREEQYNSTYRVVSVLTVLHQDWLNGKEYKCKVSNKALPAPIEKTISKAKGQPREPQVYTLPPSREEMTKNQVSLTCLVKGFYPSDIAVEWESNGQPENNYKTTPPVLDSDGSFFLYSKLTVDKSRWQQGNVFSCSVMHEALHNHYTQKSLSLSPGK

SEQ ID NO: 32 - protein, 239 aa, synthetic construct; identical to SEQ ID NO: 30

SEQ ID NO: 33 - protein, 463 aa, synthetic construct
MKHLWFFLLLVAAPRWVLSQVKLLQSGAALEKPGASVKMSCKASGYTFTDYWVIWVKQSHGKSLEWIGEIYPNSGATNFNAKFKGKATLTVDKSTSTAYMELSRLTSEDSAIYYCTTYDFDYWGQGVMVTVSSASTKGPSVFPLAPSSKSTSGGTAALGCLVKDYFPEPVTVSWNSGALTSGVHTFPAVLQSSGLYSLSSVVTVPSSSLGTQTYICNVNHKPSNTKVDKKVEPKSCDKTHTCPPCPAPELLGGPSVFLFPPKPKDTLMISRTPEVTCVVVDVSHEDPEVKFNWYVDGVEVHNAKTKPREEQYNSTYRVVSVLTVLHQDWLNGKEYKCKVSNKALPAPIEKTISKAKGQPREPQVYTLPPSREEMTKNQVSLTCLVKGFYPSDIAVEWESNGQPENNYKTTPPVLDSDGSFFLYSKLTVDKSRWQQGNVFSCSVMHEALHNHYTQKSLSLSPGK

SEQ ID NO: 34 - DNA, 717 bp, synthetic construct
  source 1..717: mol_type = other DNA
atggtgctgcagacccaggtgttcatctccctgctgctgtggatctccggcgcgtacggcgatgttgtgctgacccagactccacccactttatcggctaccattggacaatcagtctccatctcttgcaggtcaagtcagagtctctcacatactaatggaaacacctatttatattggttgctacagaggccaggccaacctccacaacttctaatttatttcgtgtccaggcttgaatctggggtccccaacaggttcagtggcagtgggtcaggaactgatttcacactcaaaatcagtggagtagaggctgaggatttgggactttattactgcgtgcaaagtacccatgttccgaacacgtttggagctgggaccaagctggaactgaaacggacggtggccgccccctccgtgttcatcttccccccctccgacgagcagctgaagtccggcaccgcctccgtggtgtgcctgctgaataacttctaccccagagaggccaaggtgcagtggaaggtggacaacgccctgcagtccgggaactcccaggagagcgtgaccgagcaggacagcaaggacagcacctacagcctgagcagcaccctgaccctgagcaaagccgactacgagaagcacaaggtgtacgcctgcgaggtgacccaccagggcctgagctcccccgtcaccaagagcttcaacaggggggagtgt

SEQ ID NO: 35 - DNA, 1389 bp, synthetic construct
  source 1..1389: mol_type = other DNA
atgaaacacctgtggttcttcctcctgctggtggcagctcccagatgggtgctgagccaggtcaagttgctgcagtctggggctgcactggagaagcctggagcctctgtgaagatgtcttgcaaagcttctggttatacattcactgactactgggtgatctgggtgaagcagagtcatggaaagagccttgagtggattggggaaatttatcctaacagtggtgctactaacttcaatgcaaagttcaagggcaaggccacattgactgtagacaaatccaccagcacagcctatatggagctcagcagattgacatctgaggactctgcaatctattactgtacaacatacgactttgattattggggccaaggagtcatggtcacagtcagctcagcctccaccaagggcccaagcgtcttccccctggcaccctcctccaagagcacctctggcggcacagccgccctgggctgcctggtcaaggactacttccccgaacccgtgaccgtgagctggaactcaggcgccctgaccagcggcgtgcacaccttccccgctgtcctgcagtcctcaggactctactccctcagcagcgtggtgaccgtgccctccagcagcttgggcacccagacctacatctgcaacgtgaatcacaagcccagcaacaccaaggtggacaagagagttgagcccaaatcttgtgacaaaactcacacatgcccaccctgcccagcacctgaagccgcggggggaccctcagtcttcctcttccccccaaaacccaaggacaccctcatgatctcccggacccctgaggtcacatgcgtggtggtggacgtgagccacgaagaccctgaggtcaagttcaactggtacgtggacggcgtggaggtgcataatgccaagacaaagccccgggaggagcagtacaacagcacgtaccgggtggtcagcgtcctcaccgtcctgcaccaggactggctgaatggcaaggagtacaagtgcaaggtctccaacaaagccctcccagcccccatcgagaaaaccatctccaaagccaaaggccagccccgggaaccacaggtgtacaccctgcccccatcccgggaggagatgaccaagaaccaggtcagcctgacctgcctggtcaaaggcttctatcccagcgacatcgccgtggagtgggagagcaatggccagcccgagaacaactacaagaccacccctcccgtgctggactccgacggctccttcttcctctacagcaagctcaccgtggacaagagcaggtggcagcagggcaacgtcttctcatgctccgtgatgcatgaggctctgcacaaccactacacccagaagagcctctccctgtctcccggcaaa

SEQ ID NO: 36 - DNA, 717 bp, synthetic construct; identical to SEQ ID NO: 34
  source 1..717: mol_type = other DNA

SEQ ID NO: 37 - DNA, 1389 bp, synthetic construct
  source 1..1389: mol_type = other DNA
atgaaacacctgtggttcttcctcctgctggtggcagctcccagatgggtgctgagccaggtcaagttgctgcagtctggggctgcactggagaagcctggagcctctgtgaagatgtcttgcaaagcttctggttatacattcactgactactgggtgatctgggtgaagcagagtcatggaaagagccttgagtggattggggaaatttatcctaacagtggtgctactaacttcaatgcaaagttcaagggcaaggccacattgactgtagacaaatccaccagcacagcctatatggagctcagcagattgacatctgaggactctgcaatctattactgtacaacatacgactttgattattggggccaaggagtcatggtcacagtcagctcagcctccaccaagggcccaagcgtcttccccctggcaccctcctccaagagcacctctggcggcacagccgccctgggctgcctggtcaaggactacttccccgaacccgtgaccgtgagctggaactcaggcgccctgaccagcggcgtgcacaccttccccgctgtcctgcagtcctcaggactctactccctcagcagcgtggtgaccgtgccctccagcagcttgggcacccagacctacatctgcaacgtgaatcacaagcccagcaacaccaaggtggacaagaaggttgagcccaaatcttgtgacaaaactcacacatgcccaccctgcccagcacctgaactcctggggggaccctcagtcttcctcttccccccaaaacccaaggacaccctcatgatctcccggacccctgaggtcacatgcgtggtggtggacgtgagccacgaagaccctgaggtcaagttcaactggtacgtggacggcgtggaggtgcataatgccaagacaaagccccgggaggagcagtacaacagcacgtaccgggtggtcagcgtcctcaccgtcctgcaccaggactggctgaatggcaaggagtacaagtgcaaggtctccaacaaagccctcccagcccccatcgagaaaaccatctccaaagccaaaggccagccccgggaaccacaggtgtacaccctgcccccatcccgggaggagatgaccaagaaccaggtcagcctgacctgcctggtcaaaggcttctatcccagcgacatcgccgtggagtgggagagcaatggccagcccgagaacaactacaagaccacccctcccgtgctggactccgacggctccttcttcctctacagcaagctcaccgtggacaagagcaggtggcagcagggcaacgtcttctcatgctccgtgatgcatgaggctctgcacaaccactacacccagaagagcctctccctgtctcccggcaaa

SEQ ID NO: 38 - DNA, 699 bp, Homo sapiens
  source 1..699: mol_type = other DNA
atggtgctgcagacccaggtgttcatctccctgctgctgtggatctccggcgcgtacggcgacatcgtgatgacacagagccctgatagcctggccgtgtctctgggagagagagccaccatcaattgcaaggccagcgagagcgtgtccaccagaatgcactggtatcagcagaagcccggccagcctcctaagctgctgatctacaaggcctccaatctggccagcggagtgcctgccagattttctggctctggcagcggcaccgatttcaccctgacaatcagttccctgcaggccgaggatgtggccgtgtactactgtcagcagagctggaatggctgggcctttggccagggcaccaaggtggaaatcaagcgtacggtggccgccccctccgtgttcatcttccccccctccgacgagcagctgaagtccggcaccgcctccgtggtgtgcctgctgaataacttctaccccagagaggccaaggtgcagtggaaggtggacaacgccctgcagtccgggaactcccaggagagcgtgaccgagcaggacagcaaggacagcacctacagcctgagcagcaccctgaccctgagcaaagccgactacgagaagcacaaggtgtacgcctgcgaggtgacccaccagggcctgagctcccccgtcaccaagagcttcaacaggggggagtgt

SEQ ID NO: 39 - DNA, 699 bp, Homo sapiens
  source 1..699: mol_type = other DNA
atggtgctgcagacccaggtgttcatctccctgctgctgtggatctccggcgcgtacggcgagatcgtgctgacacagagccctggcacactgtcactgtctccaggcgaaagagccacactgagctgcaaggccagcgagagcgtgtccacacggatgcactggtatcagcagaagcctggacaggcccctcggctgctgatctacaaggcctctaatctggccagcggcgtgccagccagattttctggttctggcagcggcaccgacttcaccctgacaatcagcagactggaacccgaggacttcgccgtgtacttctgtcagcagtcctggaacggctgggcctttggccagggaacaaaggtggaaatcaagcgtacggtggccgccccctccgtgttcatcttccccccctccgacgagcagctgaagtccggcaccgcctccgtggtgtgcctgctgaataacttctaccccagagaggccaaggtgcagtggaaggtggacaacgccctgcagtccgggaactcccaggagagcgtgaccgagcaggacagcaaggacagcacctacagcctgagcagcaccctgaccctgagcaaagccgactacgagaagcacaaggtgtacgcctgcgaggtgacccaccagggcctgagctcccccgtcaccaagagcttcaacaggggggagtgt

SEQ ID NO: 40 - DNA, 1428 bp, Homo sapiens
  source 1..1428: mol_type = other DNA
atgaaacacctgtggttcttcctcctgctggtggcagctcccagatgggtgctgagcgaggtgcagctggttgaatctggcggaggactggttcagcctggcggatctctgagactgtcttgtgccgccagcggcttcaccttcaacaactactacatggtctgggtccgacaggcccctggcaaaggacttgagtgggtcgcctacatctctaccggcggaggcaccacctactaccgcgagtctgtgaagggcagattcaccatcagccgggacaacagcaagagcaccctgtacctgcagatgaacagcctgagagccgaggacaccgccgtgtactactgtaccaccagcgtgtacttcagcgacggcagcagccactatgacggcgagtggttcgcttattggggccagggcacactggtcacagttagctcagcctccaccaagggcccaagcgtcttccccctggcaccctcctccaagagcacctctggcggcacagccgccctgggctgcctggtcaaggactacttccccgaacccgtgaccgtgagctggaactcaggcgccctgaccagcggcgtgcacaccttccccgctgtcctgcagtcctcaggactctactccctcagcagcgtggtgaccgtgccctccagcagcttgggcacccagacctacatctgcaacgtgaatcacaagcccagcaacaccaaggtggacaagaaggttgagcccaaatcttgtgacaaaactcacacatgcccaccctgcccagcacctgaactcctggggggaccctcagtcttcctcttccccccaaaacccaaggacaccctcatgatctcccggacccctgaggtcacatgcgtggtggtggacgtgagccacgaagaccctgaggtcaagttcaactggtacgtggacggcgtggaggtgcataatgccaagacaaagccccgggaggagcagtacaacagcacgtaccgggtggtcagcgtcctcaccgtcctgcaccaggactggctgaatggcaaggagtacaagtgcaaggtctccaacaaagccctcccagcccccatcgagaaaaccatctccaaagccaaaggccagccccgggaaccacaggtgtacaccctgcccccatcccgggaggagatgaccaagaaccaggtcagcctgacctgcctggtcaaaggcttctatcccagcgacatcgccgtggagtgggagagcaatggccagcccgagaacaactacaagaccacccctcccgtgctggactccgacggctccttcttcctctacagcaagctcaccgtggacaagagcaggtggcagcagggcaacgtcttctcatgctccgtgatgcatgaggctctgcacaaccactacacccagaagagcctctccctgtctcccggcaaa

SEQ ID NO: 41 - DNA, 1428 bp, Homo sapiens
  source 1..1428: mol_type = other DNA
atgaaacacctgtggttcttcctcctgctggtggcagctcccagatgggtgctgagcgaggtgcagctggttgaatctggcggaggactggttcagcctggcggatctctgagactgtcttgtgccgccagcggcttcaccttcaacaactactacatggtctgggtccgacaggcccctggcaaaggacttgagtgggtcgcctacatctctaccggcggaggcaccacctactacgccgattctgtgaagggcagattcaccatcagccgggacaacagcaagagcaccctgtacctgcagatgaacagcctgagagccgaggacaccgccgtgtactactgtaccaccagcgtgtacttcagcgacggcagcagccactatgacggcgagtggttcgcttattggggccagggcacactggtcacagttagctcagcctccaccaagggcccaagcgtcttccccctggcaccctcctccaagagcacctctggcggcacagccgccctgggctgcctggtcaaggactacttccccgaacccgtgaccgtgagctggaactcaggcgccctgaccagcggcgtgcacaccttccccgctgtcctgcagtcctcaggactctactccctcagcagcgtggtgaccgtgccctccagcagcttgggcacccagacctacatctgcaacgtgaatcacaagcccagcaacaccaaggtggacaagaaggttgagcccaaatcttgtgacaaaactcacacatgcccaccctgcccagcacctgaactcctggggggaccctcagtcttcctcttccccccaaaacccaaggacaccctcatgatctcccggacccctgaggtcacatgcgtggtggtggacgtgagccacgaagaccctgaggtcaagttcaactggtacgtggacggcgtggaggtgcataatgccaagacaaagccccgggaggagcagtacaacagcacgtaccgggtggtcagcgtcctcaccgtcctgcaccaggactggctgaatggcaaggagtacaagtgcaaggtctccaacaaagccctcccagcccccatcgagaaaaccatctccaaagccaaaggccagccccgggaaccacaggtgtacaccctgcccccatcccgggaggagatgaccaagaaccaggtcagcctgacctgcctggtcaaaggcttctatcccagcgacatcgccgtggagtgggagagcaatggccagcccgagaacaactacaagaccacccctcccgtgctggactccgacggctccttcttcctctacagcaagctcaccgtggacaagagcaggtggcagcagggcaacgtcttctcatgctccgtgatgcatgaggctctgcacaaccactacacccagaagagcctctccctgtctcccggcaaa

SEQ ID NO: 42 - DNA, 819 bp, Homo sapiens
  source 1..819: mol_type = other DNA
atggattcatacctgctgatgtggggactgctcacgttcatcatggtgcctggctgccaggcagagctctgtgacgatgacccgccagagatcccacacgccacattcaaagccatggcctacaaggaaggaaccatgttgaactgtgaatgcaagagaggtttccgcagaataaaaagcgggtcactctatatgctctgtacaggaaactctagccactcgtcctgggacaaccaatgtcaatgcacaagctctgccactcggaacacaacgaaacaagtgacacctcaacctgaagaacagaaagaaaggaaaaccacagaaatgcaaagtccaatgcagccagtggaccaagcgagccttccaggtcactgcagggaacctccaccatgggaaaatgaagccacagagagaatttatcatttcgtggtggggcagatggtttattatcagtgcgtccagggatacagggctctacacagaggtcctgctgagagcgtctgcaaaatgacccacgggaagacaaggtggacccagccccagctcatatgcacaggtgaaatggagaccagtcagtttccaggtgaagagaagcctcaggcaagccccgaaggccgtcctgagagtgagacttcctgcctcgtcacaacaacagattttcaaatacagacagaaatggctgcaaccatggagacgtccatatttacaacagagtaccaggtagcagtggccggctgtgttttcctgctgatcagcgtcctcctcctgagtgggctcacctggcagcggagacagaggaagagtagaagaacaatctag

SEQ ID NO: 43 - DNA, 807 bp, Mus musculus
  source 1..807: mol_type = other DNA
atggagccacgcttgctgatgttggggtttctctcattaaccatagtacccagttgtcgggcagaactgtgtctgtatgacccacccgaggtccccaatgccacattcaaagccctctcctacaagaacggcaccatcctaaactgtgaatgcaagagaggtttccgaagactaaaggaattggtctatatgcgttgcttaggaaactcctggagcagcaactgccagtgcaccagcaactcccatgacaaatcgagaaagcaagttacagctcaacttgaacaccagaaagagcaacaaaccacaacagacatgcagaagccaacacagtctatgcaccaagagaaccttacaggtcactgcagggagccacctccttggaaacatgaagattccaagagaatctatcatttcgtggaaggacagagtgttcactacgagtgtattccgggatacaaggctctacagagaggtcctgctattagcatctgcaagatgaagtgtgggaaaacggggtggactcagccccagctcacatgtgtagatgaaagagaacaccaccgatttctggctagtgaggaatctcaaggaagcagaaattcttctcccgagagtgagacttcctgccccataaccaccacagacttcccacaacccacagaaacaactgcaatgacggagacatttgtgctcacaatggagtataaggtagcagtggccagctgcctcttcctgctcatcagcatcctcctcctgagcgggctcacctggcaacacagatggaggaagagcagaagaaccatctag

SEQ ID NO: 44 - protein, 268 aa, Mus musculus
MEPRLLMLGFLSLTIVPSCRAELCLYDPPEVPNATFKALSYKNGTILNCECKRGFRRLKELVYMRCLGNSWSSNCQCTSNSHDKSRKQVTAQLEHQKEQQTTTDMQKPTQSMHQENLTGHCREPPPWKHEDSKRIYHFVEGQSVHYECIPGYKALQRGPAISICKMKCGKTGWTQPQLTCVDEREHHRFLASEESQGSRNSSPESETSCPITTTDFPQPTETTAMTETFVLTMEYKVAVASCLFLLISILLLSGLTWQHRWRKSRRTI

SEQ ID NO: 45 - DNA, 34 bp, synthetic construct
  source 1..34: mol_type = other DNA
ggtaccgccatggatccatacctgctcatgtggg

SEQ ID NO: 46 - DNA, 33 bp, synthetic construct
  source 1..33: mol_type = other DNA
ctcgagctagattgttcttctattcttcctctg

SEQ ID NO: 47 - DNA, 819 bp, Macaca fascicularis
  source 1..819: mol_type = other DNA
atggatccatacctgctcatgtggggactgctcacgttcatcacggtgcctggctgccaggcagagctctgtgacgatgacccgccaaaaatcacacatgccacattcaaagccgtggcctacaaggaaggaaccatgttgaactgtgaatgcaagagaggtttccgcagaataaaaagcgggtcaccctatatgctctgtacaggaaactctagccactcgtcctgggacaaccaatgtcaatgcacaagctctgctgctcggaacacaacaaaacaagtgacacctcaacctgaagaacagaaagaaagaaaaaccacagaaatgcaaagtcaaatgcagctggcggaccaagtgagccttccaggtcactgcagggaacctccaccgtgggaaaatgaagccacagaaagaatttatcatttcgtggtggggcagacggtttactaccagtgcgtccagggatacagggctctacacagaggtcctgctgagagcgtctgcaaaatgacccacgggaagacaagatggacccagccccagctcatatgcacaggtgaaacggagcccagtcagtttccaggtgaagaggagcctcaggcaagccccgacggccttcctgagagtgagacttcccgcctcgtcacaacaacagattttcgaatacagacagaagtggctgcaaccatggaaacgttcatatttacaacagagtaccaggtagcagtggccggctgtgttttcctgctgatcagcgtcctcctgctgagtgggctcacctggcagcggagacagaggaagaatagaagaacaatctag

SEQ ID NO: 48 - protein, 272 aa, Macaca fascicularis
MDPYLLMWGLLTFITVPGCQAELCDDDPPKITHATFKAVAYKEGTMLNCECKRGFRRIKSGSPYMLCTGNSSHSSWDNQCQCTSSAARNTTKQVTPQPEEQKERKTTEMQSQMQLADQVSLPGHCREPPPWENEATERIYHFVVGQTVYYQCVQGYRALHRGPAESVCKMTHGKTRWTQPQLICTGETEPSQFPGEEEPQASPDGLPESETSRLVTTTDFRIQTEVAATMETFIFTTEYQVAVAGCVFLLISVLLLSGLTWQRRQRKNRRTI

SEQ ID NO: 49 - DNA, 22 bp, synthetic construct
  source 1..22: mol_type = other DNA
agctcccagatgggtgctgagc

SEQ ID NO: 50 - DNA, 22 bp, synthetic construct
  source 1..22: mol_type = other DNA
gggcccttggtggaggctgagc

SEQ ID NO: 51 - DNA, 449 bp, synthetic construct
  source 1..449: mol_type = other DNA
gcctccggactctagagccaccatggtgctgcagacccaggtgttcatctccctgctgctgtggatctccggcgcgtacggcgatatcgtgatgattaaacgtacggtggccgccccctccgtgttcatcttccccccctccgacgagcagctgaagtccggcaccgcctccgtggtgtgcctgctgaataacttctaccccagagaggccaaggtgcagtggaaggtggacaacgccctgcagtccgggaactcccaggagagcgtgaccgagcaggacagcaaggacagcacctacagcctgagcagcaccctgaccctgagcaaagccgactacgagaagcacaaggtgtacgcctgcgaggtgacccaccagggcctgagctcccccgtcaccaagagcttcaacaggggggagtgttaggggcccgtttaaacgggggaggcta

SEQ ID NO: 52 - DNA, 1136 bp, synthetic construct
  source 1..1136: mol_type = other DNA
ccagcctccggactctagagccaccatgaaacacctgtggttcttcctcctgctggtggcagctcccagatgggtgctgagccaggtgcaattgtgcaggcggttagctcagcctccaccaagggcccaagcgtcttccccctggcaccctcctccaagagcacctctggcggcacagccgccctgggctgcctggtcaaggactacttccccgaacccgtgaccgtgagctggaactcaggcgccctgaccagcggcgtgcacaccttccccgctgtcctgcagtcctcaggactctactccctcagcagcgtggtgaccgtgccctccagcagcttgggcacccagacctacatctgcaacgtgaatcacaagcccagcaacaccaaggtggacaagagagttgagcccaaatcttgtgacaaaactcacacatgcccaccctgcccagcacctgaagccgcggggggaccctcagtcttcctcttccccccaaaacccaaggacaccctcatgatctcccggacccctgaggtcacatgcgtggtggtggacgtgagccacgaagaccctgaggtcaagttcaactggtacgtggacggcgtggaggtgcataatgccaagacaaagccccgggaggagcagtacaacagcacgtaccgggtggtcagcgtcctcaccgtcctgcaccaggactggctgaatggcaaggagtacaagtgcaaggtctccaacaaagccctcccagcccccatcgagaaaaccatctccaaagccaaaggccagccccgggaaccacaggtgtacaccctgcccccatcccgggaggagatgaccaagaaccaggtcagcctgacctgcctggtcaaaggcttctatcccagcgacatcgccgtggagtgggagagcaatggccagcccgagaacaactacaagaccacccctcccgtgctggactccgacggctccttcttcctctacagcaagctcaccgtggacaagagcaggtggcagcagggcaacgtcttctcatgctccgtgatgcatgaggctctgcacaaccactacacccagaagagcctctccctgtctcccggcaaatgagatatcgggcccgtttaaacgggggaggctaa

SEQ ID NO: 53 - DNA, 1117 bp, synthetic construct
  source 1..1117: mol_type = other DNA
gggtctagagccaccatgaaacacctgtggttcttcctcctgctggtggcagctcccagatgggtgctgagccaggtgcaattgtgcaggcggttagctcagcctccaccaagggcccaagcgtcttccccctggcaccctcctccaagagcacctctggcggcacagccgccctgggctgcctggtcaaggactacttccccgaacccgtgaccgtgagctggaactcaggcgccctgaccagcggcgtgcacaccttccccgctgtcctgcagtcctcaggactctactccctcagcagcgtggtgaccgtgccctccagcagcttgggcacccagacctacatctgcaacgtgaatcacaagcccagcaacaccaaggtggacaagaaggttgagcccaaatcttgtgacaaaactcacacatgcccaccctgcccagcacctgaactcctggggggaccctcagtcttcctcttccccccaaaacccaaggacaccctcatgatctcccggacccctgaggtcacatgcgtggtggtggacgtgagccacgaagaccctgaggtcaagttcaactggtacgtggacggcgtggaggtgcataatgccaagacaaagccccgggaggagcagtacaacagcacgtaccgggtggtcagcgtcctcaccgtcctgcaccaggactggctgaatggcaaggagtacaagtgcaaggtctccaacaaagccctcccagcccccatcgagaaaaccatctccaaagccaaaggccagccccgggaaccacaggtgtacaccctgcccccatcccgggaggagatgaccaagaaccaggtcagcctgacctgcctggtcaaaggcttctatcccagcgacatcgccgtggagtgggagagcaatggccagcccgagaacaactacaagaccacccctcccgtgctggactccgacggctccttcttcctctacagcaagctcaccgtggacaagagcaggtggcagcagggcaacgtcttctcatgctccgtgatgcatgaggctctgcacaaccactacacccagaagagcctctccctgtctcccggcaaatgagatatcgggcccgtttaaacggg

SEQ ID NO: 54 - protein, 239 aa, synthetic construct; identical to SEQ ID NO: 30

SEQ ID NO: 55 - protein, 463 aa, synthetic construct
MKHLWFFLLLVAAPRWVLSQVKLLQSGAALEKPGASVKMSCKASGYTFTDYWVIWVKQSHGKSLEWIGEIYPNSGATNFNAKFKGKATLTVDKSTSTAYMELSRLTSEDSAIYYCTTYDFDYWGQGVMVTVSSASTKGPSVFPLAPSSKSTSGGTAALGCLVKDYFPEPVTVSWNSGALTSGVHTFPAVLQSSGLYSLSSVVTVPSSSLGTQTYICNVNHKPSNTKVDKKVEPKSCDKTHTCPPCPAPEAAGGPSVFLFPPKPKDTLMISRTPEVTCVVVDVSHEDPEVKFNWYVDGVEVHNAKTKPREEQYNSTYRVVSVLTVLHQDWLNGKEYKCKVSNKALAAPIEKTISKAKGQPREPQVYTLPPSREEMTKNQVSLTCLVKGFYPSDIAVEWESNGQPENNYKTTPPVLDSDGSFFLYSKLTVDKSRWQQGNVFSCSVMHEALHNHYTQKSLSLSPGK

SEQ ID NO: 56 - DNA, 717 bp, synthetic construct; identical to SEQ ID NO: 34
  source 1..717: mol_type = other DNA

SEQ ID NO: 57 - DNA, 1389 bp, synthetic construct
  source 1..1389: mol_type = other DNA
atgaaacacctgtggttcttcctcctgctggtggcagctcccagatgggtgctgagccaggtcaagttgctgcagtctggggctgcactggagaagcctggagcctctgtgaagatgtcttgcaaagcttctggttatacattcactgactactgggtgatctgggtgaagcagagtcatggaaagagccttgagtggattggggaaatttatcctaacagtggtgctactaacttcaatgcaaagttcaagggcaaggccacattgactgtagacaaatccaccagcacagcctatatggagctcagcagattgacatctgaggactctgcaatctattactgtacaacatacgactttgattattggggccaaggagtcatggtcacagtcagctcagcctccaccaagggcccaagcgtcttccccctggcaccctcctccaagagcacctctggcggcacagccgccctgggctgcctggtcaaggactacttccccgaacccgtgaccgtgagctggaactcaggcgccctgaccagcggcgtgcacaccttccccgctgtcctgcagtcctcaggactctactccctcagcagcgtggtgaccgtgccctccagcagcttgggcacccagacctacatctgcaacgtgaatcacaagcccagcaacaccaaggtggacaagaaggttgagcccaaatcttgtgacaaaactcacacatgcccaccctgcccagcacctgaagccgcggggggaccctcagtcttcctcttccccccaaaacccaaggacaccctcatgatctcccggacccctgaggtcacatgcgtggtggtggacgtgagccacgaagaccctgaggtcaagttcaactggtacgtggacggcgtggaggtgcataatgccaagacaaagccccgggaggagcagtacaacagcacgtaccgggtggtcagcgtcctcaccgtcctgcaccaggactggctgaatggcaaggagtacaagtgcaaggtctccaacaaagccctcgcagcccccatcgagaaaaccatctccaaagccaaaggccagccccgggaaccacaggtgtacaccctgcccccatcccgggaggagatgaccaagaaccaggtcagcctgacctgcctggtcaaaggcttctatcccagcgacatcgccgtggagtgggagagcaatggccagcccgagaacaactacaagaccacccctcccgtgctggactccgacggctccttcttcctctacagcaagctcaccgtggacaagagcaggtggcagcagggcaacgtcttctcatgctccgtgatgcatgaggctctgcacaaccactacacccagaagagcctctccctgtctcccggcaaa

SEQ ID NO: 58 - DNA, 1117 bp, synthetic construct
  source 1..1117: mol_type = other DNA
gggtctagagccaccatgaaacacctgtggttcttcctcctgctggtggcagctcccagatgggtgctgagccaggtgcaattgtgcaggcggttagctcagcctccaccaagggcccaagcgtcttccccctggcaccctcctccaagagcacctctggcggcacagccgccctgggctgcctggtcaaggactacttccccgaacccgtgaccgtgagctggaactcaggcgccctgaccagcggcgtgcacaccttccccgctgtcctgcagtcctcaggactctactccctcagcagcgtggtgaccgtgccctccagcagcttgggcacccagacctacatctgcaacgtgaatcacaagcccagcaacaccaaggtggacaagaaggttgagcccaaatcttgtgacaaaactcacacatgcccaccctgcccagcacctgaagccgcggggggaccctcagtcttcctcttccccccaaaacccaaggacaccctcatgatctcccggacccctgaggtcacatgcgtggtggtggacgtgagccacgaagaccctgaggtcaagttcaactggtacgtggacggcgtggaggtgcataatgccaagacaaagccccgggaggagcagtacaacagcacgtaccgggtggtcagcgtcctcaccgtcctgcaccaggactggctgaatggcaaggagtacaagtgcaaggtctccaacaaagccctcgcagcccccatcgagaaaaccatctccaaagccaaaggccagccccgggaaccacaggtgtacaccctgcccccatcccgggaggagatgaccaagaaccaggtcagcctgacctgcctggtcaaaggcttctatcccagcgacatcgccgtggagtgggagagcaatggccagcccgagaacaactacaagaccacccctcccgtgctggactccgacggctccttcttcctctacagcaagctcaccgtggacaagagcaggtggcagcagggcaacgtcttctcatgctccgtgatgcatgaggctctgcacaaccactacacccagaagagcctctccctgtctcccggcaaatgagatatcgggcccgtttaaacggg